European Patent Specification EP 3 648 783 B1, published September 4, 2024. Title: NOVEL POLYNUCLEOTIDES ENCODING A HUMAN FKRP PROTEIN. Applicant: GENETHON UNIVERSITE D'EVRY-VAL-D'ESSONNE INSERM (INSTITUT NATIONAL DE LA SANTE ET DE LA RECHERCHE MEDICALE). The sequence listing filed with the application follows.

SEQUENCE LISTING (21 sequences)

SEQ ID NO: 1 - protein, 495 aa, Homo sapiens
  "FKRP"
  FKRP
MRLTRCQAALAAAITLNLLVLFYVSWLQHQPRNSRARGPRRASAAGPRVTVLVREFEAFDNAVPELVDSFLQQDPAQPVVVAADTLPYPPLALPRIPNVRLALLQPALDRPAAASRPETYVATEFVALVPDGARAEAPGLLERMVEALRAGSARLVAAPVATANPARCLALNVSLREWTARYGAAPAAPRCDALDGDAVVLLRARDLFNLSAPLARPVGTSLFLQTALRGWAVQLLDLTFAAARQPPLATAHARWKAEREGRARRAALLRALGIRLVSWEGGRLEWFGCNKETTRCFGTVVGDTPAYLYEERWTPPCCLRALRETARYVVGVLEAAGVRYWLEGGSLLGAARHGDIIPWDYDVDLGIYLEDVGNCEQLRGAEAGSVVDERGFVWEKAVEGDFFRVQYSESNHLHVDLWPFYPRNGVMTKDTWLDHRQDVEFPEHFLQPLVPLPFAGFVAQAPNNYRRFLELKFGPGVIENPQYPNPALLSLTGSG

SEQ ID NO: 2 - DNA, 1488 bp, Homo sapiens
  "FKRP wt"
  FKRP wt
atgcggctcacccgctgccaggctgccctggcggccgccatcaccctcaaccttctggtcctcttctatgtctcgtggctgcagcaccagcctaggaattcccgggcccgggggccccgtcgtgcctctgctgccggcccccgtgtcaccgtcctggtgcgggagttcgaggcatttgacaacgcggtgcccgagctggtagactccttcctgcagcaagacccagcccagcccgtggtggtggcagccgacacgctcccctacccgcccctggccctgccccgcatccccaacgtgcgtctggcgctgctccagcccgccctggaccggccagccgcagcctcgcgcccggagacctacgtggccaccgagtttgtggccctagtacctgatggggcgcgggctgaggcacctggcctgctggagcgcatggtggaggcgctccgcgcaggaagcgcacgtctggtggccgccccggttgccacggccaaccctgccaggtgcctggccctgaacgtcagcctgcgagagtggaccgcccgctatggcgcagcccccgccgcgccccgctgcgacgccctggacggagatgctgtggtgctcctgcgcgcccgcgacctcttcaacctctcggcgcccctggcccggccggtgggcaccagcctctttctgcagaccgcccttcgcggctgggcggtgcagctgctggacttgaccttcgccgcggcgcgccagcccccgctggccacggcccacgcgcgctggaaggctgagcgcgagggacgcgctcggcgggcggcgctgctccgcgcgctgggcatccgcctagtgagctgggaaggcgggcggctggagtggttcggctgcaacaaggagaccacgcgctgcttcggaaccgtggtgggcgacacgcccgcctacctctacgaggagcgctggacgcccccctgctgcctgcgcgcgctgcgcgagaccgcccgctatgtggtgggcgtgctggaggctgcgggcgtgcgctactggctcgagggcggctcactgctgggggccgcccgccacggggacatcatcccatgggactacgacgtggacctgggcatctacttggaggacgtgggcaactgcgagcagctgcggggggcagaggccggctcggtggtggatgagcgcggcttcgtatgggagaaggcggtcgagggcgactttttccgcgtgcagtacagcgaaagcaaccacttgcacgtggacctgtggcccttctacccccgcaatggcgtcatgaccaaggacacgtggctggaccaccggcaggatgtggagtttcccgagcacttcctgcagccgctggtgcccctgccctttgccggcttcgtggcgcaggcgcctaacaactaccgccgcttcctggagctcaagttcgggcccggggtcatcgagaacccccagtaccccaacccggcactgctgagtctgacgggaagcggctga

SEQ ID NO: 3 - DNA, 1488 bp, Artificial Sequence
  "FKRP-OPTmin"
  FKRP-OPTmin
atgcggctcacccgctgccaggctgccctggcggccgccatcaccctcaaccttctggtcctcttctatgtctcgtggctgcagcaccagcctaggaattcccgggcccgggggccccgtcgtgcctctgctgccggcccccgtgtcaccgtcctggtgcgggagttcgaggcatttgacaacgcggtgcccgagctggtagactccttcctgcagcaagacccagcccagcccgtggtggtggcagccgacacgctcccctacccgcccctggccctgccccgcatccccaacgtgcgtctggcgctgctccagcccgccctggaccggccagccgcagcctcgcgcccggagacctacgtggccaccgagtttgtggccctagtacctgatggggcgcgggctgaggcacctggcctgctggagcggatggtggaggcgctccgcgcaggaagcgcacgtctggtggccgccccggttgccacggccaaccctgccaggtgcctggccctgaacgtcagcctgcgagagtggaccgcccgctacggcgcagcccccgccgcgccccgctgcgacgccctggacggagatgctgtggtgctcctgcgcgcccgcgacctcttcaacctctcggcgcccctggcccggccggtgggcaccagcctctttctgcagaccgcccttcgcggctgggcggtgcagctgctggacttgaccttcgccgcggcgcgccagcccccgctggccacggcccacgcgcgctggaaggctgagcgcgagggacgcgctcggcgggcggcgctgctccgcgcgctgggaatccgcctagtgagctgggaaggcgggcggctggagtggttcggctgcaacaaggagaccacgcgctgcttcggaaccgtggtgggcgacacgcccgcctacctctacgaggagcgctggacgcccccctgctgcctgcgcgcgctgcgcgagaccgcccgctatgtggtgggcgtgctggaggctgcgggcgtgcgctactggctcgagggcggctcactgctgggggccgcccgccacggggacatcatcccatgggactacgacgtggacctgggcatctacttggaggacgtgggcaactgcgagcagctgcggggggcagaggccggctcggtggtggatgagcgcggcttcgtatgggagaaggcggtcgagggcgactttttccgcgtgcagtacagcgaaagcaaccacttgcacgtggacctgtggcccttctacccccgcaatggcgtcatgaccaaggacacgtggctggaccaccggcaggatgtggagtttcccgagcacttcctgcagccgctggtgcccctgccctttgccggcttcgtggcgcaggcgcctaacaactaccgccgcttcctggagctcaagttcgggcccggggtgatcgagaacccccagtaccccaacccggcactgctgagtctgacgggaagcggctga

SEQ ID NO: 4 - DNA, 1488 bp, Artificial Sequence
  "FKRP-OPTcomp"
  FKRP-OPTcomp
atgagactgaccaggtgccaggctgccctggctgctgccatcaccctgaacctgctggtgctgttctatgtgagctggctgcagcaccagcccaggaacagcagggccaggggccccaggagggcctctgctgctggccccagggtgacagtgctggtgagggagtttgaggcctttgacaatgctgtgcctgagctggtggacagcttcctgcagcaggaccctgcccagcctgtggtggtggctgctgataccctgccctacccccccctggccctgcccaggatccccaatgtgaggctggccctgctgcagcctgccctggacaggcctgctgctgccagcaggcctgagacctatgtggccacagagtttgtggccctggtgcctgatggggccagggctgaggcccctggcctgctggagaggatggtggaggccctgagggctggctctgccaggctggtggctgcccctgtggccacagccaaccctgccaggtgcctggccctgaatgtgagcctgagagagtggacagccaggtatggggctgcccctgctgcccccaggtgtgatgccctggatggagatgctgtggtgctgctgagggccagggacctgttcaacctgtctgcccccctggccaggcctgtggggaccagcctgtttctgcagacagccctgaggggctgggctgtgcagctgctggacctgacctttgctgctgccaggcagccccccctggctacagcccacgccaggtggaaggctgagagggagggcagggccaggagggctgccctgctgagggccctggggatcaggctggtgagctgggaggggggcaggctggagtggtttggctgcaacaaggagacaaccaggtgctttgggacagtggtgggggatacccctgcctacctgtatgaggagaggtggacccccccctgctgcctgagggccctgagggagacagccaggtatgtggtgggggtgctggaggctgctggggtgaggtactggctggaggggggcagcctgctgggggctgccaggcacggggacattatcccctgggactatgatgtggacctgggcatctacctggaggatgtgggcaactgtgagcagctgaggggggctgaggctggctctgtggtggatgagaggggctttgtgtgggagaaggctgtggagggggactttttcagggtgcagtactctgagagcaaccacctgcacgtggacctgtggcccttctaccccaggaatggggtgatgaccaaggacacctggctggaccacaggcaggatgtggagttccctgagcacttcctgcagcccctggtgcccctgccctttgctggctttgtggcccaggcccccaacaactacaggaggttcctggagctgaagtttggccctggggtgattgagaacccccagtaccccaaccctgccctgctgagcctgacaggctctggctga

SEQ ID NO: 5 - DNA, 1488 bp, Artificial Sequence
  "FKRP-OPT-07"
  FKRP-OPT-07
atgcggctcacccgctgccaggctgccctggctgccgccatcaccctcaaccttctggtcctcttctatgtcagctggctgcagcaccagcctaggaattcccgggcccgggggcccaggagggcctctgctgccggccccagggtcaccgtcctggtgcgggagttcgaggcatttgacaacgctgtgcccgagctggtagactccttcctgcagcaagacccagcccagcccgtggtggtggcagccgacaccctcccctacccccccctggccctgccccgcatccccaacgtgaggctggccctgctccagcccgccctggaccggccagccgcagccagccgccctgagacctacgtggccaccgagtttgtggccctggtacctgatggggcccgggctgaggcacctggcctgctggagcggatggtggaggccctccgcgcaggaagcgcaaggctggtggccgcccctgttgccacagccaaccctgccaggtgcctggccctgaacgtcagcctgcgagagtggaccgcccgctacggcgcagcccccgccgccccccgctgcgacgccctggacggagatgctgtggtgctcctgcgcgcccgcgacctcttcaacctctctgcccccctggcccggcctgtgggcaccagcctctttctgcagaccgcccttcgcggctgggctgtgcagctgctggacttgaccttcgccgctgcccgccagccccccctggccacagcccacgcccgctggaaggctgagcgcgagggacgcgctcggcgggctgccctgctccgcgccctgggaatccgcctggtgagctgggaaggcgggcggctggagtggttcggctgcaacaaggagaccacccgctgcttcggaaccgtggtgggcgacacccccgcctacctctacgaggagcgctggacccccccctgctgcctgcgcgccctgcgcgagaccgcccgctatgtggtgggcgtgctggaggctgctggcgtgcgctactggctcgagggcggctcactgctgggggccgcccgccacggggacatcatcccatgggactacgacgtggacctgggcatctacttggaggacgtgggcaactgcgagcagctgcggggggcagaggccggctctgtggtggatgagcgcggcttcgtatgggagaaggctgtcgagggcgactttttccgcgtgcagtacagcgaaagcaaccacttgcacgtggacctgtggcccttctacccccgcaatggcgtcatgaccaaggacacctggctggaccaccggcaggatgtggagtttcccgagcacttcctgcagcccctggtgcccctgccctttgccggcttcgtggcccaggcccctaacaactaccgccgcttcctggagctcaagttcgggcccggggtgatcgagaacccccagtaccccaaccctgcactgctgagtctgaccggaagcggctga

SEQ ID NO: 6 - DNA, 1488 bp, Artificial Sequence
  "FKRP-OPT-08"
  FKRP-OPT-08
atgcggctcacccgctgccaggctgccctggctgctgccatcaccctcaaccttctggtcctcttctatgtcagctggctgcagcaccagcctaggaattcccgggcccgggggcccaggagggcctctgctgctggccccagggtcaccgtcctggtgcgggagttcgaggcatttgacaacgctgtgcccgagctggtagactccttcctgcagcaagacccagcccagcccgtggtggtggcagctgacaccctcccctacccccccctggccctgccccgcatccccaacgtgaggctggccctgctccagcccgccctggaccggccagctgcagccagccgccctgagacctacgtggccaccgagtttgtggccctggtacctgatggggcccgggctgaggcacctggcctgctggagcggatggtggaggccctcagggcaggaagcgcaaggctggtggctgcccctgttgccacagccaaccctgccaggtgcctggccctgaacgtcagcctgcgagagtggaccgcccgctacggggcagcccccgctgccccccgctgcgacgccctggacggagatgctgtggtgctcctgagggccagggacctcttcaacctctctgcccccctggcccggcctgtgggcaccagcctctttctgcagaccgcccttaggggctgggctgtgcagctgctggacttgaccttcgctgctgcccgccagccccccctggccacagcccacgcccgctggaaggctgagagggagggaagggctcggcgggctgccctgctcagggccctgggaatccgcctggtgagctgggaaggggggcggctggagtggttcggctgcaacaaggagaccacccgctgcttcggaaccgtggtgggggacacccccgcctacctctacgaggagcgctggacccccccctgctgcctgagggccctgagggagaccgcccgctatgtggtgggggtgctggaggctgctggggtgcgctactggctcgaggggggctcactgctgggggctgcccgccacggggacatcatcccatgggactacgacgtggacctgggcatctacttggaggacgtgggcaactgcgagcagctgcggggggcagaggctggctctgtggtggatgagaggggcttcgtatgggagaaggctgtggagggggactttttcagggtgcagtacagcgaaagcaaccacttgcacgtggacctgtggcccttctacccccgcaatggggtcatgaccaaggacacctggctggaccaccggcaggatgtggagtttcccgagcacttcctgcagcccctggtgcccctgccctttgctggcttcgtggcccaggcccctaacaactaccgccgcttcctggagctcaagttcgggcccggggtgatcgagaacccccagtaccccaaccctgcactgctgagtctgaccggaagcggctga

SEQ ID NO: 7 - DNA, 1488 bp, Artificial Sequence
  "FKRP-OPT-10"
  FKRP-OPT-10
atgagactgacaaggtgccaggctgccctggctgctgccatcacactgaacctgctggtgctgttttatgtgagctggctgcagcaccagcctaggaacagcagggccaggggccctaggagggcctctgctgctggccctagggtgacagtgctggtgagggagtttgaggcctttgacaatgctgtgcctgagctggtggacagctttctgcagcaggaccctgcccagcctgtggtggtggctgctgatacactgccttaccctcctctggccctgcctaggatccctaatgtgaggctggccctgctgcagcctgccctggacaggcctgctgctgccagcaggcctgagacttatgtggccacagagtttgtggccctggtgcctgatggggccagggctgaggcccctggcctgctggagaggatggtggaggccctgagggctggctctgccaggctggtggctgcccctgtggccacagccaaccctgccaggtgcctggccctgaatgtgagcctgagagagtggacagccaggtatggggctgcccctgctgcccctaggtgtgatgccctggatggagatgctgtggtgctgctgagggccagggacctgtttaacctgtctgcccctctggccaggcctgtggggacaagcctgtttctgcagacagccctgaggggctgggctgtgcagctgctggacctgacatttgctgctgccaggcagcctcctctggctacagcccacgccaggtggaaggctgagagggagggcagggccaggagggctgccctgctgagggccctggggatcaggctggtgagctgggaggggggcaggctggagtggtttggctgcaacaaggagacaacaaggtgctttgggacagtggtgggggatacacctgcctacctgtatgaggagaggtggacacctccttgctgcctgagggccctgagggagacagccaggtatgtggtgggggtgctggaggctgctggggtgaggtactggctggaggggggcagcctgctgggggctgccaggcacggggacattatcccttgggactatgatgtggacctgggcatctacctggaggatgtgggcaactgtgagcagctgaggggggctgaggctggctctgtggtggatgagaggggctttgtgtgggagaaggctgtggagggggacttttttagggtgcagtactctgagagcaaccacctgcacgtggacctgtggcctttttaccctaggaatggggtgatgacaaaggacacatggctggaccacaggcaggatgtggagtttcctgagcactttctgcagcctctggtgcctctgccttttgctggctttgtggcccaggcccctaacaactacaggaggtttctggagctgaagtttggccctggggtgattgagaaccctcagtaccctaaccctgccctgctgagcctgacaggctctggctga

SEQ ID NO: 8 - DNA, 1488 bp, Artificial Sequence
  "FKRP-OPT-11"
  FKRP-OPT-11
atgagactgacaaggtgccaggctgccctggctgctgccatcacactgaacctgctggtgctgttttatgtgagctggctgcagcaccagcctagaaacagcagagccagaggccctagaagagcctctgctgctggccctagagtgacagtgctggtgagagagtttgaggcctttgacaatgctgtgcctgagctggtggacagctttctgcagcaggaccctgcccagcctgtggtggtggctgctgatacactgccttaccctcctctggccctgcctagaatccctaatgtgagactggccctgctgcagcctgccctggacagacctgctgctgccagcagacctgagacttatgtggccacagagtttgtggccctggtgcctgatggggccagagctgaggcccctggcctgctggagagaatggtggaggccctgagagctggctctgccagactggtggctgcccctgtggccacagccaaccctgccagatgcctggccctgaatgtgagcctgagagagtggacagccagatatggggctgcccctgctgcccctagatgtgatgccctggatggagatgctgtggtgctgctgagagccagagacctgtttaacctgtctgcccctctggccagacctgtggggacaagcctgtttctgcagacagccctgagaggctgggctgtgcagctgctggacctgacatttgctgctgccagacagcctcctctggctacagcccacgccagatggaaggctgagagagagggcagagccagaagagctgccctgctgagagccctggggatcaggctggtgagctgggaggggggcagactggagtggtttggctgcaacaaggagacaacaagatgctttgggacagtggtgggggatacacctgcctacctgtatgaggagaggtggacacctccttgctgcctgagagccctgagagagacagccagatatgtggtgggggtgctggaggctgctggggtgagatactggctggaggggggcagcctgctgggggctgccagacacggggacattatcccttgggactatgatgtggacctgggcatctacctggaggatgtgggcaactgtgagcagctgagaggggctgaggctggctctgtggtggatgagagaggctttgtgtgggagaaggctgtggagggggacttttttagagtgcagtactctgagagcaaccacctgcacgtggacctgtggcctttttaccctagaaatggggtgatgacaaaggacacatggctggaccacagacaggatgtggagtttcctgagcactttctgcagcctctggtgcctctgccttttgctggctttgtggcccaggcccctaacaactacagaagatttctggagctgaagtttggccctggggtgattgagaaccctcagtaccctaaccctgccctgctgagcctgacaggctctggctga

SEQ ID NO: 9 - DNA, 6903 bp, Artificial Sequence
  "pAAV-hDesmin-hFKRPwt"
  pAAV-hDesmin-hFKRPwt
tcgcgcgtttcggtgatgacggtgaaaacctctgacacatgcagctcccggagacggtcacagcttgtctgtaagcggatgccgggagcagacaagcccgtcagggcgcgtcagcgggtgttggcgggtgtcggggctggcttaactatgcggcatcagagcagattgtactgagagtgcaccatatgcggtgtgaaataccgcacagatgcgtaaggagaaaataccgcatcaggcgccattcgccattcaggctgcgcaactgttgggaagggcgatcggtgcgggcctcttcgctattacgccagctggcgaaagggggatgtgctgcaaggcgattaagttgggtaacgccagggttttcccagtcacgacgttgtaaaacgacggccagtgaattcgagctcggtaccttaaaccggttcctacatatgggttgcgcaatgcggccgcagtactgcagaaataggccgaaatcggcaaaatccctttattggccactccctctctgcgcgctcgctcgctcactgaggccgggcgaccaaaggtcgcccgacgcccgggctttgcccgggcggcctcagtgagcgagcgagcgcgcagagagggagtggccaactccatcactaggggttccttaccccctgccccccacagctcctctcctgtgccttgtttcccagccatgcgttctcctctataaatacccgctctggtatttggggttggcagctgttgctgccagggagatggttgggttgacatgcggctcctgacaaaacacaaacccctggtgtgtgtgggcgtgggtggtgtgagtagggggatgaatcagggagggggcgggggacccagggggcaggagccacacaaagtctgtgcgggggtgggagcgcacatagcaattggaaactgaaagcttatcagaccctttctggaaatcagcccactgtttataaacttgaggccccaccctcgacagtaccggggaggaagagggcctgcactagtccagagggaaactgaggctcagggctagctcgcccatagacatacatggcaggcaggctttggccaggatccctccgcctgccaggcgtctccctgccctcccttcctgcctagagacccccaccctcaagcctggctggtctttgcctgagacccaaacctcttcgacttcaagagaatatttaggaacaaggtggtttagggcctttcctgggaacaggccttgaccctttaagaaatgacccaaagtctctccttgaccaaaaaggggaccctcaaactaaagggaagcctctcttctgctgtctcccctgaccccactcccccccaccccaggacgaggagataaccagggctgaaagaggcccgcctgggggctgcagacatgcttgctgcctgccctggcgaaggattggcaggcttgcccgtcacaggacccccgctggctgactcaggggcgcaggcctcttgcgggggagctggcctccccgcccccacggccacgggccgccctttcctggcaggacagcgggatcttgcagctgtcaggggaggggaggcgggggctgatgtcaggagggatacaaatagtgccgacggctgggggccctgtctcccctcgccgcatccactctccggccggccgcctgcccgccgcctcctccgtgcgcccgccagcctcgcccgcgtacacatattgaccaaatcagggtaattttgcatttgtaattttaaaaaatgctttcttcttttaatatacttttttgtttatcttatttctaatactttccctaatctctttctttcagggcaataatgatacaatgtatcatgcctctttgcaccattctaaagaataacagtgataatttctgggttaaggcaatagcaatatttctgcatataaatatttctgcatataaattgtaactgatgtaagaggtttcatattgctaatagcagctacaatccagctaccattctgcttttattttttggttgggataaggctggattattctgagtccaagctaggcccttttgctaatcttgttcatacctcttatcttcctcccacagctcctgggcaacgtgctggtctctgtgctggcccatcactttggcaaagaattcgccaccatgcggctcacccgctgccaggctgccctggcggccgccatcaccctcaaccttctggtcctcttctatgtctcgtggctgcagcaccagcctaggaattcccgggcccgggggccccgtcgtgcctctgctgccggcccccgtgtcaccgtcctggtgcgggagttcgaggcatttgacaacgcggtgcccgagctggtagactccttcctgcagcaagacccagcccagcccgtggtggtggcagccgacacgctcccctacccgcccctggccctgccccgcatccccaacgtgcgtctggcgctgctccagcccgccctggaccggccagccgcagcctcgcgcccggagacctacgtggccaccgagtttgtggccctagtacctgatggggcgcgggctgaggcacctggcctgctggagcgcatggtggaggcgctccgcgcaggaagcgcacgtctggtggccgccccggttgccacggccaaccctgccaggtgcctggccctgaacgtcagcctgcgagagtggaccgcccgctatggcgcagcccccgccgcgccccgctgcgacgccctggacggagatgctgtggtgctcctgcgcgcccgcgacctcttcaacctctcggcgcccctggcccggccggtgggcaccagcctctttctgcagaccgcccttcgcggctgggcggtgcagctgctggacttgaccttcgccgcggcgcgccagcccccgctggccacggcccacgcgcgctggaaggctgagcgcgagggacgcgctcggcgggcggcgctgctccgcgcgctgggcatccgcctagtgagctgggaaggcgggcggctggagtggttcggctgcaacaaggagaccacgcgctgcttcggaaccgtggtgggcgacacgcccgcctacctctacgaggagcgctggacgcccccctgctgcctgcgcgcgctgcgcgagaccgcccgctatgtggtgggcgtgctggaggctgcgggcgtgcgctactggctcgagggcggctcactgctgggggccgcccgccacggggacatcatcccatgggactacgacgtggacctgggcatctacttggaggacgtgggcaactgcgagcagctgcggggggcagaggccggctcggtggtggatgagcgcggcttcgtatgggagaaggcggtcgagggcgactttttccgcgtgcagtacagcgaaagcaaccacttgcacgtggacctgtggcccttctacccccgcaatggcgtcatgaccaaggacacgtggctggaccaccggcaggatgtggagtttcccgagcacttcctgcagccgctggtgcccctgccctttgccggcttcgtggcgcaggcgcctaacaactaccgccgcttcctggagctcaagttcgggcccggggtcatcgagaacccccagtaccccaacccggcactgctgagtctgacgggaagcggctgaattcaccccaccagtgcaggctgcctatcagaaagtggtggctggtgtggctaatgccctggcccacaagtatcactaagctcgctttcttgctgtccaatttctattaaaggttcctttgttccctaagtccaactactaaactgggggatattatgaagggccttgagcatctggattctgcctaataaaaaacatttattttcattgcaatgatgtatttaaattatttctgaatattttactaaaaagggaatgtgggaggtcagtgcatttaaaacataaagaaatgaagagctagttcaaaccttgggaaaatacactatatcttaaactccatgaaagaaggtgaggctgcaaacagctaatgcacattggcaacagccctgatgcctatgccttattcatccctcagaaaaggattcaagtagaggcttgatttggaggttaaagttttgctatgctgtattttacattacttattgttttagctgtcctcatgaatgtcttttcactacccatttgcttatcctgcatctctcagccttgactccactcagttctcttgcttagagataccacctttcccctgaagtgttccttccatgttttacggcgagatggtttctcctcgcctggccactcagccttagttgtctctgttgtcttatagaggtctacttgaagaaggaaaaacagggggcatggtttgactgtcctgtgagcccttcttccctgcctcccccactcacagtgacccggaatcaggaacccctagtgatggagttggccactccctctctgcgcgctcgctcgctcactgaggccgggcgaccaaaggtcgcccgacgcccgggctttgcccgggcggcctcagtgagcgagcgagcgcgcagagagggagtggccaatttgagttcttctactcaggttaaacttaagcgcggccgcagtcctaggttgcgcaatgggcatgctacagatcttccgcggtgcagcaagtcgactgcagaggcctgcatgcaagcttggcgtaatcatggtcatagctgtttcctgtgtgaaattgttatccgctcacaattccacacaacatacgagccggaagcataaagtgtaaagcctggggtgcctaatgagtgagctaactcacattaattgcgttgcgctcactgcccgctttccagtcgggaaacctgtcgtgccagctgcattaatgaatcggccaacgcgcggggagaggcggtttgcgtattgggcgctcttccgcttcctcgctcactgactcgctgcgctcggtcgttcggctgcggcgagcggtatcagctcactcaaaggcggtaatacggttatccacagaatcaggggataacgcaggaaagaacatgtgagcaaaaggccagcaaaaggccaggaaccgtaaaaaggccgcgttgctggcgtttttccataggctccgcccccctgacgagcatcacaaaaatcgacgctcaagtcagaggtggcgaaacccgacaggactataaagataccaggcgtttccccctggaagctccctcgtgcgctctcctgttccgaccctgccgcttaccggatacctgtccgcctttctcccttcgggaagcgtggcgctttctcatagctcacgctgtaggtatctcagttcggtgtaggtcgttcgctccaagctgggctgtgtgcacgaaccccccgttcagcccgaccgctgcgccttatccggtaactatcgtcttgagtccaacccggtaagacacgacttatcgccactggcagcagccactggtaacaggattagcagagcgaggtatgtaggcggtgctacagagttcttgaagtggtggcctaactacggctacactagaagaacagtatttggtatctgcgctctgctgaagccagttaccttcggaaaaagagttggtagctcttgatccggcaaacaaaccaccgctggtagcggtggtttttttgtttgcaagcagcagattacgcgcagaaaaaaaggatctcaagaagatcctttgatcttttctacggggtctgacgctcagtggaacgaaaactcacgttaagggattttggtcatgagattatcaaaaaggatcttcacctagatccttttaaattaaaaatgaagttttaaatcaatctaaagtatatatgagtaaacttggtctgacagttaccaatgcttaatcagtgaggcacctatctcagcgatctgtctatttcgttcatccatagttgcctgactccccgtcgtgtagataactacgatacgggagggcttaccatctggccccagtgctgcaatgataccgcgagacccacgctcaccggctccagatttatcagcaataaaccagccagccggaagggccgagcgcagaagtggtcctgcaactttatccgcctccatccagtctattaattgttgccgggaagctagagtaagtagttcgccagttaatagtttgcgcaacgttgttgccattgctacaggcatcgtggtgtcacgctcgtcgtttggtatggcttcattcagctccggttcccaacgatcaaggcgagttacatgatcccccatgttgtgcaaaaaagcggttagctccttcggtcctccgatcgttgtcagaagtaagttggccgcagtgttatcactcatggttatggcagcactgcataattctcttactgtcatgccatccgtaagatgcttttctgtgactggtgagtactcaaccaagtcattctgagaatagtgtatgcggcgaccgagttgctcttgcccggcgtcaatacgggataataccgcgccacatagcagaactttaaaagtgctcatcattggaaaacgttcttcggggcgaaaactctcaaggatcttaccgctgttgagatccagttcgatgtaacccactcgtgcacccaactgatcttcagcatcttttactttcaccagcgtttctgggtgagcaaaaacaggaaggcaaaatgccgcaaaaaagggaataagggcgacacggaaatgttgaatactcatactcttcctttttcaatattattgaagcatttatcagggttattgtctcatgagcggatacatatttgaatgtatttagaaaaataaacaaataggggttccgcgcacatttccccgaaaagtgccacctgacgtctaagaaaccattattatcatgacattaacctataaaaataggcgtatcacgaggccctttcgtc

SEQ ID NO: 10 - DNA, 6903 bp, Artificial Sequence
  "pAAV-hDesmin-hFKRP-OPTmin "
  pAAV-hDesmin-hFKRP-OPTmin
tcgcgcgtttcggtgatgacggtgaaaacctctgacacatgcagctcccggagacggtcacagcttgtctgtaagcggatgccgggagcagacaagcccgtcagggcgcgtcagcgggtgttggcgggtgtcggggctggcttaactatgcggcatcagagcagattgtactgagagtgcaccatatgcggtgtgaaataccgcacagatgcgtaaggagaaaataccgcatcaggcgccattcgccattcaggctgcgcaactgttgggaagggcgatcggtgcgggcctcttcgctattacgccagctggcgaaagggggatgtgctgcaaggcgattaagttgggtaacgccagggttttcccagtcacgacgttgtaaaacgacggccagtgaattcgagctcggtaccttaaaccggttcctacatatgggttgcgcaatgcggccgcagtactgcagaaataggccgaaatcggcaaaatccctttattggccactccctctctgcgcgctcgctcgctcactgaggccgggcgaccaaaggtcgcccgacgcccgggctttgcccgggcggcctcagtgagcgagcgagcgcgcagagagggagtggccaactccatcactaggggttccttaccccctgccccccacagctcctctcctgtgccttgtttcccagccatgcgttctcctctataaatacccgctctggtatttggggttggcagctgttgctgccagggagatggttgggttgacatgcggctcctgacaaaacacaaacccctggtgtgtgtgggcgtgggtggtgtgagtagggggatgaatcagggagggggcgggggacccagggggcaggagccacacaaagtctgtgcgggggtgggagcgcacatagcaattggaaactgaaagcttatcagaccctttctggaaatcagcccactgtttataaacttgaggccccaccctcgacagtaccggggaggaagagggcctgcactagtccagagggaaactgaggctcagggctagctcgcccatagacatacatggcaggcaggctttggccaggatccctccgcctgccaggcgtctccctgccctcccttcctgcctagagacccccaccctcaagcctggctggtctttgcctgagacccaaacctcttcgacttcaagagaatatttaggaacaaggtggtttagggcctttcctgggaacaggccttgaccctttaagaaatgacccaaagtctctccttgaccaaaaaggggaccctcaaactaaagggaagcctctcttctgctgtctcccctgaccccactcccccccaccccaggacgaggagataaccagggctgaaagaggcccgcctgggggctgcagacatgcttgctgcctgccctggcgaaggattggcaggcttgcccgtcacaggacccccgctggctgactcaggggcgcaggcctcttgcgggggagctggcctccccgcccccacggccacgggccgccctttcctggcaggacagcgggatcttgcagctgtcaggggaggggaggcgggggctgatgtcaggagggatacaaatagtgccgacggctgggggccctgtctcccctcgccgcatccactctccggccggccgcctgcccgccgcctcctccgtgcgcccgccagcctcgcccgcgtacacatattgaccaaatcagggtaattttgcatttgtaattttaaaaaatgctttcttcttttaatatacttttttgtttatcttatttctaatactttccctaatctctttctttcagggcaataatgatacaatgtatcatgcctctttgcaccattctaaagaataacagtgataatttctgggttaaggcaatagcaatatttctgcatataaatatttctgcatataaattgtaactgatgtaagaggtttcatattgctaatagcagctacaatccagctaccattctgcttttattttttggttgggataaggctggattattctgagtccaagctaggcccttttgctaatcttgttcatacctcttatcttcctcccacagctcctgggcaacgtgctggtctctgtgctggcccatcactttggcaaagaattcgccaccatgcggctcacccgctgccaggctgccctggcggccgccatcaccctcaaccttctggtcctcttctatgtctcgtggctgcagcaccagcctaggaattcccgggcccgggggccccgtcgtgcctctgctgccggcccccgtgtcaccgtcctggtgcgggagttcgaggcatttgacaacgcggtgcccgagctggtagactccttcctgcagcaagacccagcccagcccgtggtggtggcagccgacacgctcccctacccgcccctggccctgccccgcatccccaacgtgcgtctggcgctgctccagcccgccctggaccggccagccgcagcctcgcgcccggagacctacgtggccaccgagtttgtggccctagtacctgatggggcgcgggctgaggcacctggcctgctggagcggatggtggaggcgctccgcgcaggaagcgcacgtctggtggccgccccggttgccacggccaaccctgccaggtgcctggccctgaacgtcagcctgcgagagtggaccgcccgctacggcgcagcccccgccgcgccccgctgcgacgccctggacggagatgctgtggtgctcctgcgcgcccgcgacctcttcaacctctcggcgcccctggcccggccggtgggcaccagcctctttctgcagaccgcccttcgcggctgggcggtgcagctgctggacttgaccttcgccgcggcgcgccagcccccgctggccacggcccacgcgcgctggaaggctgagcgcgagggacgcgctcggcgggcggcgctgctccgcgcgctgggaatccgcctagtgagctgggaaggcgggcggctggagtggttcggctgcaacaaggagaccacgcgctgcttcggaaccgtggtgggcgacacgcccgcctacctctacgaggagcgctggacgcccccctgctgcctgcgcgcgctgcgcgagaccgcccgctatgtggtgggcgtgctggaggctgcgggcgtgcgctactggctcgagggcggctcactgctgggggccgcccgccacggggacatcatcccatgggactacgacgtggacctgggcatctacttggaggacgtgggcaactgcgagcagctgcggggggcagaggccggctcggtggtggatgagcgcggcttcgtatgggagaaggcggtcgagggcgactttttccgcgtgcagtacagcgaaagcaaccacttgcacgtggacctgtggcccttctacccccgcaatggcgtcatgaccaaggacacgtggctggaccaccggcaggatgtggagtttcccgagcacttcctgcagccgctggtgcccctgccctttgccggcttcgtggcgcaggcgcctaacaactaccgccgcttcctggagctcaagttcgggcccggggtgatcgagaacccccagtaccccaacccggcactgctgagtctgacgggaagcggctgaattcaccccaccagtgcaggctgcctatcagaaagtggtggctggtgtggctaatgccctggcccacaagtatcactaagctcgctttcttgctgtccaatttctattaaaggttcctttgttccctaagtccaactactaaactgggggatattatgaagggccttgagcatctggattctgcctaataaaaaacatttattttcattgcaatgatgtatttaaattatttctgaatattttactaaaaagggaatgtgggaggtcagtgcatttaaaacataaagaaatgaagagctagttcaaaccttgggaaaatacactatatcttaaactccatgaaagaaggtgaggctgcaaacagctaatgcacattggcaacagccctgatgcctatgccttattcatccctcagaaaaggattcaagtagaggcttgatttggaggttaaagttttgctatgctgtattttacattacttattgttttagctgtcctcatgaatgtcttttcactacccatttgcttatcctgcatctctcagccttgactccactcagttctcttgcttagagataccacctttcccctgaagtgttccttccatgttttacggcgagatggtttctcctcgcctggccactcagccttagttgtctctgttgtcttatagaggtctacttgaagaaggaaaaacagggggcatggtttgactgtcctgtgagcccttcttccctgcctcccccactcacagtgacccggaatcaggaacccctagtgatggagttggccactccctctctgcgcgctcgctcgctcactgaggccgggcgaccaaaggtcgcccgacgcccgggctttgcccgggcggcctcagtgagcgagcgagcgcgcagagagggagtggccaatttgagttcttctactcaggttaaacttaagcgcggccgcagtcctaggttgcgcaatgggcatgctacagatcttccgcggtgcagcaagtcgactgcagaggcctgcatgcaagcttggcgtaatcatggtcatagctgtttcctgtgtgaaattgttatccgctcacaattccacacaacatacgagccggaagcataaagtgtaaagcctggggtgcctaatgagtgagctaactcacattaattgcgttgcgctcactgcccgctttccagtcgggaaacctgtcgtgccagctgcattaatgaatcggccaacgcgcggggagaggcggtttgcgtattgggcgctcttccgcttcctcgctcactgactcgctgcgctcggtcgttcggctgcggcgagcggtatcagctcactcaaaggcggtaatacggttatccacagaatcaggggataacgcaggaaagaacatgtgagcaaaaggccagcaaaaggccaggaaccgtaaaaaggccgcgttgctggcgtttttccataggctccgcccccctgacgagcatcacaaaaatcgacgctcaagtcagaggtggcgaaacccgacaggactataaagataccaggcgtttccccctggaagctccctcgtgcgctctcctgttccgaccctgccgcttaccggatacctgtccgcctttctcccttcgggaagcgtggcgctttctcatagctcacgctgtaggtatctcagttcggtgtaggtcgttcgctccaagctgggctgtgtgcacgaaccccccgttcagcccgaccgctgcgccttatccggtaactatcgtcttgagtccaacccggtaagacacgacttatcgccactggcagcagccactggtaacaggattagcagagcgaggtatgtaggcggtgctacagagttcttgaagtggtggcctaactacggctacactagaagaacagtatttggtatctgcgctctgctgaagccagttaccttcggaaaaagagttggtagctcttgatccggcaaacaaaccaccgctggtagcggtggtttttttgtttgcaagcagcagattacgcgcagaaaaaaaggatctcaagaagatcctttgatcttttctacggggtctgacgctcagtggaacgaaaactcacgttaagggattttggtcatgagattatcaaaaaggatcttcacctagatccttttaaattaaaaatgaagttttaaatcaatctaaagtatatatgagtaaacttggtctgacagttaccaatgcttaatcagtgaggcacctatctcagcgatctgtctatttcgttcatccatagttgcctgactccccgtcgtgtagataactacgatacgggagggcttaccatctggccccagtgctgcaatgataccgcgagacccacgctcaccggctccagatttatcagcaataaaccagccagccggaagggccgagcgcagaagtggtcctgcaactttatccgcctccatccagtctattaattgttgccgggaagctagagtaagtagttcgccagttaatagtttgcgcaacgttgttgccattgctacaggcatcgtggtgtcacgctcgtcgtttggtatggcttcattcagctccggttcccaacgatcaaggcgagttacatgatcccccatgttgtgcaaaaaagcggttagctccttcggtcctccgatcgttgtcagaagtaagttggccgcagtgttatcactcatggttatggcagcactgcataattctcttactgtcatgccatccgtaagatgcttttctgtgactggtgagtactcaaccaagtcattctgagaatagtgtatgcggcgaccgagttgctcttgcccggcgtcaatacgggataataccgcgccacatagcagaactttaaaagtgctcatcattggaaaacgttcttcggggcgaaaactctcaaggatcttaccgctgttgagatccagttcgatgtaacccactcgtgcacccaactgatcttcagcatcttttactttcaccagcgtttctgggtgagcaaaaacaggaaggcaaaatgccgcaaaaaagggaataagggcgacacggaaatgttgaatactcatactcttcctttttcaatattattgaagcatttatcagggttattgtctcatgagcggatacatatttgaatgtatttagaaaaataaacaaataggggttccgcgcacatttccccgaaaagtgccacctgacgtctaagaaaccattattatcatgacattaacctataaaaataggcgtatcacgaggccctttcgtc

SEQ ID NO: 11 - DNA, 6903 bp, Artificial Sequence
  "pAAV-hDesmin-hFKRP-OPTcomp"
  pAAV-hDesmin-hFKRP-OPTcomp
tcgcgcgtttcggtgatgacggtgaaaacctctgacacatgcagctcccggagacggtcacagcttgtctgtaagcggatgccgggagcagacaagcccgtcagggcgcgtcagcgggtgttggcgggtgtcggggctggcttaactatgcggcatcagagcagattgtactgagagtgcaccatatgcggtgtgaaataccgcacagatgcgtaaggagaaaataccgcatcaggcgccattcgccattcaggctgcgcaactgttgggaagggcgatcggtgcgggcctcttcgctattacgccagctggcgaaagggggatgtgctgcaaggcgattaagttgggtaacgccagggttttcccagtcacgacgttgtaaaacgacggccagtgaattcgagctcggtaccttaaaccggttcctacatatgggttgcgcaatgcggccgcagtactgcagaaataggccgaaatcggcaaaatccctttattggccactccctctctgcgcgctcgctcgctcactgaggccgggcgaccaaaggtcgcccgacgcccgggctttgcccgggcggcctcagtgagcgagcgagcgcgcagagagggagtggccaactccatcactaggggttccttaccccctgccccccacagctcctctcctgtgccttgtttcccagccatgcgttctcctctataaatacccgctctggtatttggggttggcagctgttgctgccagggagatggttgggttgacatgcggctcctgacaaaacacaaacccctggtgtgtgtgggcgtgggtggtgtgagtagggggatgaatcagggagggggcgggggacccagggggcaggagccacacaaagtctgtgcgggggtgggagcgcacatagcaattggaaactgaaagcttatcagaccctttctggaaatcagcccactgtttataaacttgaggccccaccctcgacagtaccggggaggaagagggcctgcactagtccagagggaaactgaggctcagggctagctcgcccatagacatacatggcaggcaggctttggccaggatccctccgcctgccaggcgtctccctgccctcccttcctgcctagagacccccaccctcaagcctggctggtctttgcctgagacccaaacctcttcgacttcaagagaatatttaggaacaaggtggtttagggcctttcctgggaacaggccttgaccctttaagaaatgacccaaagtctctccttgaccaaaaaggggaccctcaaactaaagggaagcctctcttctgctgtctcccctgaccccactcccccccaccccaggacgaggagataaccagggctgaaagaggcccgcctgggggctgcagacatgcttgctgcctgccctggcgaaggattggcaggcttgcccgtcacaggacccccgctggctgactcaggggcgcaggcctcttgcgggggagctggcctccccgcccccacggccacgggccgccctttcctggcaggacagcgggatcttgcagctgtcaggggaggggaggcgggggctgatgtcaggagggatacaaatagtgccgacggctgggggccctgtctcccctcgccgcatccactctccggccggccgcctgcccgccgcctcctccgtgcgcccgccagcctcgcccgcgtacacatattgaccaaatcagggtaattttgcatttgtaattttaaaaaatgctttcttcttttaatatacttttttgtttatcttatttctaatactttccctaatctctttctttcagggcaataatgatacaatgtatcatgcctctttgcaccattctaaagaataacagtgataatttctgggttaaggcaatagcaatatttctgcatataaatatttctgcatataaattgtaactgatgtaagaggtttcatattgctaatagcagctacaatccagctaccattctgcttttattttttggttgggataaggctggattattctgagtccaagctaggcccttttgctaatcttgttcatacctcttatcttcctcccacagctcctgggcaacgtgctggtctctgtgctggcccatcactttggcaaagaattcgccaccatgagactgaccaggtgccaggctgccctggctgctgccatcaccctgaacctgctggtgctgttctatgtgagctggctgcagcaccagcccaggaacagcagggccaggggccccaggagggcctctgctgctggccccagggtgacagtgctggtgagggagtttgaggcctttgacaatgctgtgcctgagctggtggacagcttcctgcagcaggaccctgcccagcctgtggtggtggctgctgataccctgccctacccccccctggccctgcccaggatccccaatgtgaggctggccctgctgcagcctgccctggacaggcctgctgctgccagcaggcctgagacctatgtggccacagagtttgtggccctggtgcctgatggggccagggctgaggcccctggcctgctggagaggatggtggaggccctgagggctggctctgccaggctggtggctgcccctgtggccacagccaaccctgccaggtgcctggccctgaatgtgagcctgagagagtggacagccaggtatggggctgcccctgctgcccccaggtgtgatgccctggatggagatgctgtggtgctgctgagggccagggacctgttcaacctgtctgcccccctggccaggcctgtggggaccagcctgtttctgcagacagccctgaggggctgggctgtgcagctgctggacctgacctttgctgctgccaggcagccccccctggctacagcccacgccaggtggaaggctgagagggagggcagggccaggagggctgccctgctgagggccctggggatcaggctggtgagctgggaggggggcaggctggagtggtttggctgcaacaaggagacaaccaggtgctttgggacagtggtgggggatacccctgcctacctgtatgaggagaggtggacccccccctgctgcctgagggccctgagggagacagccaggtatgtggtgggggtgctggaggctgctggggtgaggtactggctggaggggggcagcctgctgggggctgccaggcacggggacattatcccctgggactatgatgtggacctgggcatctacctggaggatgtgggcaactgtgagcagctgaggggggctgaggctggctctgtggtggatgagaggggctttgtgtgggagaaggctgtggagggggactttttcagggtgcagtactctgagagcaaccacctgcacgtggacctgtggcccttctaccccaggaatggggtgatgaccaaggacacctggctggaccacaggcaggatgtggagttccctgagcacttcctgcagcccctggtgcccctgccctttgctggctttgtggcccaggcccccaacaactacaggaggttcctggagctgaagtttggccctggggtgattgagaacccccagtaccccaaccctgccctgctgagcctgacaggctctggctgaattcaccccaccagtgcaggctgcctatcagaaagtggtggctggtgtggctaatgccctggcccacaagtatcactaagctcgctttcttgctgtccaatttctattaaaggttcctttgttccctaagtccaactactaaactgggggatattatgaagggccttgagcatctggattctgcctaataaaaaacatttattttcattgcaatgatgtatttaaattatttctgaatattttactaaaaagggaatgtgggaggtcagtgcatttaaaacataaagaaatgaagagctagttcaaaccttgggaaaatacactatatcttaaactccatgaaagaaggtgaggctgcaaacagctaatgcacattggcaacagccctgatgcctatgccttattcatccctcagaaaaggattcaagtagaggcttgatttggaggttaaagttttgctatgctgtattttacattacttattgttttagctgtcctcatgaatgtcttttcactacccatttgcttatcctgcatctctcagccttgactccactcagttctcttgcttagagataccacctttcccctgaagtgttccttccatgttttacggcgagatggtttctcctcgcctggccactcagccttagttgtctctgttgtcttatagaggtctacttgaagaaggaaaaacagggggcatggtttgactgtcctgtgagcccttcttccctgcctcccccactcacagtgacccggaatcaggaacccctagtgatggagttggccactccctctctgcgcgctcgctcgctcactgaggccgggcgaccaaaggtcgcccgacgcccgggctttgcccgggcggcctcagtgagcgagcgagcgcgcagagagggagtggccaatttgagttcttctactcaggttaaacttaagcgcggccgcagtcctaggttgcgcaatgggcatgctacagatcttccgcggtgcagcaagtcgactgcagaggcctgcatgcaagcttggcgtaatcatggtcatagctgtttcctgtgtgaaattgttatccgctcacaattccacacaacatacgagccggaagcataaagtgtaaagcctggggtgcctaatgagtgagctaactcacattaattgcgttgcgctcactgcccgctttccagtcgggaaacctgtcgtgccagctgcattaatgaatcggccaacgcgcggggagaggcggtttgcgtattgggcgctcttccgcttcctcgctcactgactcgctgcgctcggtcgttcggctgcggcgagcggtatcagctcactcaaaggcggtaatacggttatccacagaatcaggggataacgcaggaaagaacatgtgagcaaaaggccagcaaaaggccaggaaccgtaaaaaggccgcgttgctggcgtttttccataggctccgcccccctgacgagcatcacaaaaatcgacgctcaagtcagaggtggcgaaacccgacaggactataaagataccaggcgtttccccctggaagctccctcgtgcgctctcctgttccgaccctgccgcttaccggatacctgtccgcctttctcccttcgggaagcgtggcgctttctcatagctcacgctgtaggtatctcagttcggtgtaggtcgttcgctccaagctgggctgtgtgcacgaaccccccgttcagcccgaccgctgcgccttatccggtaactatcgtcttgagtccaacccggtaagacacgacttatcgccactggcagcagccactggtaacaggattagcagagcgaggtatgtaggcggtgctacagagttcttgaagtggtggcctaactacggctacactagaagaacagtatttggtatctgcgctctgctgaagccagttaccttcggaaaaagagttggtagctcttgatccggcaaacaaaccaccgctggtagcggtggtttttttgtttgcaagcagcagattacgcgcagaaaaaaaggatctcaagaagatcctttgatcttttctacggggtctgacgctcagtggaacgaaaactcacgttaagggattttggtcatgagattatcaaaaaggatcttcacctagatccttttaaattaaaaatgaagttttaaatcaatctaaagtatatatgagtaaacttggtctgacagttaccaatgcttaatcagtgaggcacctatctcagcgatctgtctatttcgttcatccatagttgcctgactccccgtcgtgtagataactacgatacgggagggcttaccatctggccccagtgctgcaatgataccgcgagacccacgctcaccggctccagatttatcagcaataaaccagccagccggaagggccgagcgcagaagtggtcctgcaactttatccgcctccatccagtctattaattgttgccgggaagctagagtaagtagttcgccagttaatagtttgcgcaacgttgttgccattgctacaggcatcgtggtgtcacgctcgtcgtttggtatggcttcattcagctccggttcccaacgatcaaggcgagttacatgatcccccatgttgtgcaaaaaagcggttagctccttcggtcctccgatcgttgtcagaagtaagttggccgcagtgttatcactcatggttatggcagcactgcataattctcttactgtcatgccatccgtaagatgcttttctgtgactggtgagtactcaaccaagtcattctgagaatagtgtatgcggcgaccgagttgctcttgcccggcgtcaatacgggataataccgcgccacatagcagaactttaaaagtgctcatcattggaaaacgttcttcggggcgaaaactctcaaggatcttaccgctgttgagatccagttcgatgtaacccactcgtgcacccaactgatcttcagcatcttttactttcaccagcgtttctgggtgagcaaaaacaggaaggcaaaatgccgcaaaaaagggaataagggcgacacggaaatgttgaatactcatactcttcctttttcaatattattgaagcatttatcagggttattgtctcatgagcggatacatatttgaatgtatttagaaaaataaacaaataggggttccgcgcacatttccccgaaaagtgccacctgacgtctaagaaaccattattatcatgacattaacctataaaaataggcgtatcacgaggccctttcgtc

SEQ ID NO: 12 - DNA, 145 bp, Artificial Sequence
  "ITR 5'"
  ITR 5'
ttggccactccctctctgcgcgctcgctcgctcactgaggccgggcgaccaaaggtcgcccgacgcccgggctttgcccgggcggcctcagtgagcgagcgagcgcgcagagagggagtggccaactccatcactaggggttcct

SEQ ID NO: 13 - DNA, 1061 bp, Artificial Sequence
  "human desmin promoter"
  human desmin promoter
taccccctgccccccacagctcctctcctgtgccttgtttcccagccatgcgttctcctctataaatacccgctctggtatttggggttggcagctgttgctgccagggagatggttgggttgacatgcggctcctgacaaaacacaaacccctggtgtgtgtgggcgtgggtggtgtgagtagggggatgaatcagggagggggcgggggacccagggggcaggagccacacaaagtctgtgcgggggtgggagcgcacatagcaattggaaactgaaagcttatcagaccctttctggaaatcagcccactgtttataaacttgaggccccaccctcgacagtaccggggaggaagagggcctgcactagtccagagggaaactgaggctcagggctagctcgcccatagacatacatggcaggcaggctttggccaggatccctccgcctgccaggcgtctccctgccctcccttcctgcctagagacccccaccctcaagcctggctggtctttgcctgagacccaaacctcttcgacttcaagagaatatttaggaacaaggtggtttagggcctttcctgggaacaggccttgaccctttaagaaatgacccaaagtctctccttgaccaaaaaggggaccctcaaactaaagggaagcctctcttctgctgtctcccctgaccccactcccccccaccccaggacgaggagataaccagggctgaaagaggcccgcctgggggctgcagacatgcttgctgcctgccctggcgaaggattggcaggcttgcccgtcacaggacccccgctggctgactcaggggcgcaggcctcttgcgggggagctggcctccccgcccccacggccacgggccgccctttcctggcaggacagcgggatcttgcagctgtcaggggaggggaggcgggggctgatgtcaggagggatacaaatagtgccgacggctgggggccctgtctcccctcgccgcatccactctccggccggccgcctgcccgccgcctcctccgtgcgcccgccagcctcgcccgc

SEQ ID NO: 14 - DNA, 452 bp, Artificial Sequence
  "HBB2 intron followed by Kozak sequence"
  HBB2 intron followed by Kozak sequence
gtacacatattgaccaaatcagggtaattttgcatttgtaattttaaaaaatgctttcttcttttaatatacttttttgtttatcttatttctaatactttccctaatctctttctttcagggcaataatgatacaatgtatcatgcctctttgcaccattctaaagaataacagtgataatttctgggttaaggcaatagcaatatttctgcatataaatatttctgcatataaattgtaactgatgtaagaggtttcatattgctaatagcagctacaatccagctaccattctgcttttattttttggttgggataaggctggattattctgagtccaagctaggcccttttgctaatcttgttcatacctcttatcttcctcccacagctcctgggcaacgtgctggtctctgtgctggcccatcactttggcaaagaattcgccacc

SEQ ID NO: 15 - DNA, 766 bp, Artificial Sequence
  "HBB2 polyA"
  HBB2 polyA
attcaccccaccagtgcaggctgcctatcagaaagtggtggctggtgtggctaatgccctggcccacaagtatcactaagctcgctttcttgctgtccaatttctattaaaggttcctttgttccctaagtccaactactaaactgggggatattatgaagggccttgagcatctggattctgcctaataaaaaacatttattttcattgcaatgatgtatttaaattatttctgaatattttactaaaaagggaatgtgggaggtcagtgcatttaaaacataaagaaatgaagagctagttcaaaccttgggaaaatacactatatcttaaactccatgaaagaaggtgaggctgcaaacagctaatgcacattggcaacagccctgatgcctatgccttattcatccctcagaaaaggattcaagtagaggcttgatttggaggttaaagttttgctatgctgtattttacattacttattgttttagctgtcctcatgaatgtcttttcactacccatttgcttatcctgcatctctcagccttgactccactcagttctcttgcttagagataccacctttcccctgaagtgttccttccatgttttacggcgagatggtttctcctcgcctggccactcagccttagttgtctctgttgtcttatagaggtctacttgaagaaggaaaaacagggggcatggtttgactgtcctgtgagcccttcttccctgcctcccccactcacagtgacccggaatc

SEQ ID NO: 16 - DNA, 145 bp, Artificial Sequence
  "ITR 3’"
  ITR 3’
aggaacccctagtgatggagttggccactccctctctgcgcgctcgctcgctcactgaggccgggcgaccaaaggtcgcccgacgcccgggctttgcccgggcggcctcagtgagcgagcgagcgcgcagagagggagtggccaa

SEQ ID NO: 17 - DNA, 18 bp, Artificial Sequence
  "Forward HBB2 polyA "
  Forward HBB2 polyA
ccaggcgaggagaaacca

SEQ ID NO: 18 - DNA, 25 bp, Artificial Sequence
  "Reverse HBB2 polyA "
  Reverse HBB2 polyA
cttgactccactcagttctcttgct

SEQ ID NO: 19 - DNA, 29 bp, Artificial Sequence
  "Probe HBB2 polyA "
  Probe HBB2 polyA
ctcgccgtaaaacatggaaggaacacttc

SEQ ID NO: 20 - DNA, 1488 bp, Artificial Sequence
  "WO2016/138387 (FKRP-06)"
  WO2016/138387 (FKRP-06)
atgagactgacaagatgccaggccgccctggccgctgccatcacactgaatctgctggtgctgttctatgtgtcctggctgcagcaccagccccggaactctagagccagaggcccaagaagggcctctgccgccggacctagagtgacagtgctcgtgcgcgagttcgaggccttcgacaatgccgtgcccgagctggtggacagcttcctgcagcaagaccctgctcagcctgtggtggtggccgccgatacactgccttatcctccactggccctgcccagaatccccaatgtgcgactggctctgctgcagcccgccctggatagacctgccgccgctagcagacctgagacatacgtggccaccgagttcgtggccctggtgcctgatggcgccagagctgaagctcccggcctgctggaaagaatggtggaagccctgagagccggcagcgccagactggtggctgctcctgtggctaccgccaaccctgccagatgtctggccctgaatgtgtccctgagagagtggaccgccagatacggcgctgcccctgccgctcctagatgtgatgctctggatggcgacgccgtggtgctgctgagagccagggacctgttcaacctgagcgcccctctggccagacctgtgggcacaagcctgtttctgcagacagccctgaggggctgggccgtgcagctgctggatctgacatttgccgctgccagacagcctcctctggccacagcccatgccagatggaaggccgagagagagggcagagccagaagggctgctctgctgagggccctgggcatcagactggtgtcttgggaaggcggcagactcgagtggttcggctgcaacaaagaaaccacccggtgcttcggcaccgtcgtgggcgatacaccagcctacctgtacgaggaaagatggacccccccttgctgcctgcgggccctgagagaaacagccagatatgtcgtgggcgtgctggaagccgctggcgtgcgatattggctggaaggcggatctctgctgggagccgccaggcacggcgacatcatcccttgggactacgacgtggacctgggcatctacctggaagatgtgggcaactgcgagcagctgagaggcgccgaagccggctctgtggtggatgagaggggcttcgtgtgggagaaggccgtggaaggcgacttcttccgggtgcagtacagcgagagcaaccatctgcatgtggacctgtggcccttctacccccggaacggcgtgatgaccaaggacacctggctggaccaccggcaggacgtggaattccccgagcactttctgcagcccctggtgccactgcctttcgccggatttgtggcccaggcccccaacaactaccggcggttcctggaactgaagttcggccctggcgtgatcgagaacccccagtaccctaaccctgccctgctgagcctgaccggcagcggctaa

SEQ ID NO: 21 - DNA, 6903 bp, Artificial Sequence
  "pAAV-hDesmin-hFKRP-OPT08"
  pAAV-hDesmin-hFKRP-OPT08
tcgcgcgtttcggtgatgacggtgaaaacctctgacacatgcagctcccggagacggtcacagcttgtctgtaagcggatgccgggagcagacaagcccgtcagggcgcgtcagcgggtgttggcgggtgtcggggctggcttaactatgcggcatcagagcagattgtactgagagtgcaccatatgcggtgtgaaataccgcacagatgcgtaaggagaaaataccgcatcaggcgccattcgccattcaggctgcgcaactgttgggaagggcgatcggtgcgggcctcttcgctattacgccagctggcgaaagggggatgtgctgcaaggcgattaagttgggtaacgccagggttttcccagtcacgacgttgtaaaacgacggccagtgaattcgagctcggtaccttaaaccggttcctacatatgggttgcgcaatgcggccgcagtactgcagaaataggccgaaatcggcaaaatccctttattggccactccctctctgcgcgctcgctcgctcactgaggccgggcgaccaaaggtcgcccgacgcccgggctttgcccgggcggcctcagtgagcgagcgagcgcgcagagagggagtggccaactccatcactaggggttccttaccccctgccccccacagctcctctcctgtgccttgtttcccagccatgcgttctcctctataaatacccgctctggtatttggggttggcagctgttgctgccagggagatggttgggttgacatgcggctcctgacaaaacacaaacccctggtgtgtgtgggcgtgggtggtgtgagtagggggatgaatcagggagggggcgggggacccagggggcaggagccacacaaagtctgtgcgggggtgggagcgcacatagcaattggaaactgaaagcttatcagaccctttctggaaatcagcccactgtttataaacttgaggccccaccctcgacagtaccggggaggaagagggcctgcactagtccagagggaaactgaggctcagggctagctcgcccatagacatacatggcaggcaggctttggccaggatccctccgcctgccaggcgtctccctgccctcccttcctgcctagagacccccaccctcaagcctggctggtctttgcctgagacccaaacctcttcgacttcaagagaatatttaggaacaaggtggtttagggcctttcctgggaacaggccttgaccctttaagaaatgacccaaagtctctccttgaccaaaaaggggaccctcaaactaaagggaagcctctcttctgctgtctcccctgaccccactcccccccaccccaggacgaggagataaccagggctgaaagaggcccgcctgggggctgcagacatgcttgctgcctgccctggcgaaggattggcaggcttgcccgtcacaggacccccgctggctgactcaggggcgcaggcctcttgcgggggagctggcctccccgcccccacggccacgggccgccctttcctggcaggacagcgggatcttgcagctgtcaggggaggggaggcgggggctgatgtcaggagggatacaaatagtgccgacggctgggggccctgtctcccctcgccgcatccactctccggccggccgcctgcccgccgcctcctccgtgcgcccgccagcctcgcccgcgtacacatattgaccaaatcagggtaattttgcatttgtaattttaaaaaatgctttcttcttttaatatacttttttgtttatcttatttctaatactttccctaatctctttctttcagggcaataatgatacaatgtatcatgcctctttgcaccattctaaagaataacagtgataatttctgggttaaggcaatagcaatatttctgcatataaatatttctgcatataaattgtaactgatgtaagaggtttcatattgctaatagcagctacaatccagctaccattctgcttttattttttggttgggataaggctggattattctgagtccaagctaggcccttttgctaatcttgttcatacctcttatcttcctcccacagctcctgggcaacgtgctggtctctgtgctggcccatcactttggcaaagaattcgccaccatgcggctcacccgctgccaggctgccctggctgctgccatcaccctcaaccttctggtcctcttctatgtcagctggctgcagcaccagcctaggaattcccgggcccgggggcccaggagggcctctgctgctggccccagggtcaccgtcctggtgcgggagttcgaggcatttgacaacgctgtgcccgagctggtagactccttcctgcagcaagacccagcccagcccgtggtggtggcagctgacaccctcccctacccccccctggccctgccccgcatccccaacgtgaggctggccctgctccagcccgccctggaccggccagctgcagccagccgccctgagacctacgtggccaccgagtttgtggccctggtacctgatggggcccgggctgaggcacctggcctgctggagcggatggtggaggccctcagggcaggaagcgcaaggctggtggctgcccctgttgccacagccaaccctgccaggtgcctggccctgaacgtcagcctgcgagagtggaccgcccgctacggggcagcccccgctgccccccgctgcgacgccctggacggagatgctgtggtgctcctgagggccagggacctcttcaacctctctgcccccctggcccggcctgtgggcaccagcctctttctgcagaccgcccttaggggctgggctgtgcagctgctggacttgaccttcgctgctgcccgccagccccccctggccacagcccacgcccgctggaaggctgagagggagggaagggctcggcgggctgccctgctcagggccctgggaatccgcctggtgagctgggaaggggggcggctggagtggttcggctgcaacaaggagaccacccgctgcttcggaaccgtggtgggggacacccccgcctacctctacgaggagcgctggacccccccctgctgcctgagggccctgagggagaccgcccgctatgtggtgggggtgctggaggctgctggggtgcgctactggctcgaggggggctcactgctgggggctgcccgccacggggacatcatcccatgggactacgacgtggacctgggcatctacttggaggacgtgggcaactgcgagcagctgcggggggcagaggctggctctgtggtggatgagaggggcttcgtatgggagaaggctgtggagggggactttttcagggtgcagtacagcgaaagcaaccacttgcacgtggacctgtggcccttctacccccgcaatggggtcatgaccaaggacacctggctggaccaccggcaggatgtggagtttcccgagcacttcctgcagcccctggtgcccctgccctttgctggcttcgtggcccaggcccctaacaactaccgccgcttcctggagctcaagttcgggcccggggtgatcgagaacccccagtaccccaaccctgcactgctgagtctgaccggaagcggctgaattcaccccaccagtgcaggctgcctatcagaaagtggtggctggtgtggctaatgccctggcccacaagtatcactaagctcgctttcttgctgtccaatttctattaaaggttcctttgttccctaagtccaactactaaactgggggatattatgaagggccttgagcatctggattctgcctaataaaaaacatttattttcattgcaatgatgtatttaaattatttctgaatattttactaaaaagggaatgtgggaggtcagtgcatttaaaacataaagaaatgaagagctagttcaaaccttgggaaaatacactatatcttaaactccatgaaagaaggtgaggctgcaaacagctaatgcacattggcaacagccctgatgcctatgccttattcatccctcagaaaaggattcaagtagaggcttgatttggaggttaaagttttgctatgctgtattttacattacttattgttttagctgtcctcatgaatgtcttttcactacccatttgcttatcctgcatctctcagccttgactccactcagttctcttgcttagagataccacctttcccctgaagtgttccttccatgttttacggcgagatggtttctcctcgcctggccactcagccttagttgtctctgttgtcttatagaggtctacttgaagaaggaaaaacagggggcatggtttgactgtcctgtgagcccttcttccctgcctcccccactcacagtgacccggaatcaggaacccctagtgatggagttggccactccctctctgcgcgctcgctcgctcactgaggccgggcgaccaaaggtcgcccgacgcccgggctttgcccgggcggcctcagtgagcgagcgagcgcgcagagagggagtggccaatttgagttcttctactcaggttaaacttaagcgcggccgcagtcctaggttgcgcaatgggcatgctacagatcttccgcggtgcagcaagtcgactgcagaggcctgcatgcaagcttggcgtaatcatggtcatagctgtttcctgtgtgaaattgttatccgctcacaattccacacaacatacgagccggaagcataaagtgtaaagcctggggtgcctaatgagtgagctaactcacattaattgcgttgcgctcactgcccgctttccagtcgggaaacctgtcgtgccagctgcattaatgaatcggccaacgcgcggggagaggcggtttgcgtattgggcgctcttccgcttcctcgctcactgactcgctgcgctcggtcgttcggctgcggcgagcggtatcagctcactcaaaggcggtaatacggttatccacagaatcaggggataacgcaggaaagaacatgtgagcaaaaggccagcaaaaggccaggaaccgtaaaaaggccgcgttgctggcgtttttccataggctccgcccccctgacgagcatcacaaaaatcgacgctcaagtcagaggtggcgaaacccgacaggactataaagataccaggcgtttccccctggaagctccctcgtgcgctctcctgttccgaccctgccgcttaccggatacctgtccgcctttctcccttcgggaagcgtggcgctttctcatagctcacgctgtaggtatctcagttcggtgtaggtcgttcgctccaagctgggctgtgtgcacgaaccccccgttcagcccgaccgctgcgccttatccggtaactatcgtcttgagtccaacccggtaagacacgacttatcgccactggcagcagccactggtaacaggattagcagagcgaggtatgtaggcggtgctacagagttcttgaagtggtggcctaactacggctacactagaagaacagtatttggtatctgcgctctgctgaagccagttaccttcggaaaaagagttggtagctcttgatccggcaaacaaaccaccgctggtagcggtggtttttttgtttgcaagcagcagattacgcgcagaaaaaaaggatctcaagaagatcctttgatcttttctacggggtctgacgctcagtggaacgaaaactcacgttaagggattttggtcatgagattatcaaaaaggatcttcacctagatccttttaaattaaaaatgaagttttaaatcaatctaaagtatatatgagtaaacttggtctgacagttaccaatgcttaatcagtgaggcacctatctcagcgatctgtctatttcgttcatccatagttgcctgactccccgtcgtgtagataactacgatacgggagggcttaccatctggccccagtgctgcaatgataccgcgagacccacgctcaccggctccagatttatcagcaataaaccagccagccggaagggccgagcgcagaagtggtcctgcaactttatccgcctccatccagtctattaattgttgccgggaagctagagtaagtagttcgccagttaatagtttgcgcaacgttgttgccattgctacaggcatcgtggtgtcacgctcgtcgtttggtatggcttcattcagctccggttcccaacgatcaaggcgagttacatgatcccccatgttgtgcaaaaaagcggttagctccttcggtcctccgatcgttgtcagaagtaagttggccgcagtgttatcactcatggttatggcagcactgcataattctcttactgtcatgccatccgtaagatgcttttctgtgactggtgagtactcaaccaagtcattctgagaatagtgtatgcggcgaccgagttgctcttgcccggcgtcaatacgggataataccgcgccacatagcagaactttaaaagtgctcatcattggaaaacgttcttcggggcgaaaactctcaaggatcttaccgctgttgagatccagttcgatgtaacccactcgtgcacccaactgatcttcagcatcttttactttcaccagcgtttctgggtgagcaaaaacaggaaggcaaaatgccgcaaaaaagggaataagggcgacacggaaatgttgaatactcatactcttcctttttcaatattattgaagcatttatcagggttattgtctcatgagcggatacatatttgaatgtatttagaaaaataaacaaataggggttccgcgcacatttccccgaaaagtgccacctgacgtctaagaaaccattattatcatgacattaacctataaaaataggcgtatcacgaggccctttcgtc